European Patent Application EP 4 806 907 A1, published September 16, 2026. Title: MOLECULA DE ACIDO NUCLEICO RECOMBINANTE, EPITOPO DE ALFA TOXINA DE C. NOVYI RECOMBINANTE E SEU USO, VETOR DE EXPRESSAO, COMPOSICAO VACINAL, METODO PARA PREVENIR OU TRATAR CLOSTRIDIOSES EM UM INDIVIDUO SOFRENDO DO MESMO E METODO PARA PRODUZIR UMA COMPOSIÇÃO VACINAL CONTRA CLOSTRIDIOSE. Applicant: FUNDAÇÃO OSWALDO CRUZ. Application WO. The sequence listing filed with the application follows.

SEQUENCE LISTING (4 sequences)

SEQ ID NO: 1 - DNA, 279 bp, C. novyi
  source 1..279: mol_type = genomic DNA
atcaaaaacacctttgatatgctgagcagccagaatcaagaaatttttgaagccagcaacaacctgtactttagcaaaacccatgatgagtttaaaagcagctggctgctgcgtagtaatattgccgaaaaagaatttcagaaactgatcaaaacctacattggtcgcaccctgaattatgaagatggcctgaatttcaacaaatggaaacgtgttaccacctccgaactgctgaaagttattgaagaagttaacagcaccaaaatctatgaaaattat

SEQ ID NO: 2 - protein, 93 aa, C. novyi
IKNTFDMLSSQNQEIFEASNNLYFSKTHDEFKSSWLLRSNIAEKEFQKLIKTYIGRTLNYEDGLNFNKWKRVTTSELLKVIEEVNSTKIYENY

SEQ ID NO: 3 - DNA, 543 bp, C. novyi
  source 1..543: mol_type = genomic DNA
gttagcggtgttgatgaaaataatcgctatctggaatatatgctgagcaccaacaacaagtggattattaacggtggctattgggagaacgatttcaacaactataaaatcgtggactttgaaaaatgcaacgtgattgttagcggcagcaataaactgaatagcgaaggtgatctggcagataccattgatgttctggataaagatctggaaaacctgtatatcgatagcgtgattattatcccgaaagtgtacaccaagaaaatcatcattcatccgattccgaataacccgcagattaacattattaacacccagagcatccacgataaatgccatctgattattgatagcgtgctgaccaataactatcattgggaaagtgatggtgatgacctgattattaccaatggcctggatattaacattcgcattctgcagggtctgagctttggctttaaatacaaaaacatctatctgaaattcagcaactacgatgaactgagcctgaacgattttctgctgcagaattataacgtgaaa

SEQ ID NO: 4 - protein, 181 aa, C. novyi
VSGVDENNRYLEYMLSTNNKWIINGGYWENDFNNYKIVDFEKCNVIVSGSNKLNSEGDLADTIDVLDKDLENLYIDSVIIIPKVYTKKIIIHPIPNNPQINIINTQSIHDKCHLIIDSVLTNNYHWESDGDDLIITNGLDINIRILQGLSFGFKYKNIYLKFSNYDELSLNDFLLQNYNVK